European Patent Specification EP 3 772 905 B1, published February 18, 2026. Title: FAD2 GENES AND MUTATIONS. Applicant: Cibus US LLC Cibus Europe, B.V. Application Not Yet Assigned. The sequence listing filed with the application follows.

SEQUENCE LISTING (54 sequences)

SEQ ID NO: 1 - DNA, 1155 bp, Brassica napus
atgggtgcaggtggaagaatgcaagtgtctcctccctccaaaaagtctgaaaccgacaacatcaagcgcgtaccctgcgagacaccgcccttcactgtcggagaactcaagaaagcaatcccaccgcactgtttcaaacgctcgatccctcgctctttctcctacctcatctgggacatcatcatagcctcctgcttctactacgtcgccaccacttacttccctctcctccctcaccctctctcctacttcgcctggcctctctactgggcctgccagggctgcgtcctaaccggcgtctgggtcatagcccacgagtgcggccaccacgccttcagcgactaccagtggctggacgacaccgtcggcctcatcttccactccttcctcctcgtcccttacttctcctggaagtacagtcatcgacgccaccattccaacactggctccctcgagagagacgaagtgtttgtccccaagaagaagtcagacatcaagtggtacggcaagtacctcaacaaccctttgggacgcaccgtgatgttaacggttcagttcactctcggctggcctttgtacttagccttcaacgtctcggggagaccttacgacggcggcttcgcttgccatttccaccccaacgctcccatctacaacgaccgtgagcgtctccagatatacatctccgacgctggcatcctcgccgtctgctacggtctctaccgctacgctgctgtccaaggagttgcctcgatggtctgcttctacggagttcctcttctgattgtcaacgggttcttagttttgatcacttacttgcagcacacgcatccttccctgcctcactatgactcgtctgagtgggattggttgaggggagctttggccaccgttgacagagactacggaatcttgaacaaggtcttccacaatatcacggacacgcacgtggcgcatcacctgttctcgaccatgccgcattatcatgcgatggaagctacgaaggcgataaagccgatactgggagagtattatcagttcgatgggacgccggtggttaaggcgatgtggagggaggcgaaggagtgtatctatgtggaaccggacaggcaaggtgagaagaaaggtgtgttctggtacaacaataagttatga

SEQ ID NO: 2 - DNA, 1155 bp, Brassica napus
atgggtgcaggtggaagaatgcaagtgtctcctccctccaagaagtctgaaaccgacaccatcaagcgcgtaccctgcgagacaccgcccttcactgtcggagaactcaagaaagcaatcccaccgcactgtttcaaacgctcgatccctcgctctttctcctacctcatctgggacatcatcatagcctcctgcttctactacgtcgccaccacttacttccctctcctccctcaccctctctcctacttcgcctggcctctctactgggcctgccaagggtgcgtcctaaccggcgtctgggtcatagcccacgagtgcggccaccacgccttcagcgactaccagtggcttgacgacaccgtcggtctcatcttccactccttcctcctcgtcccttacttctcctggaagtacagtcatcgacgccaccattccaacactggctccctcgagagagacgaagtgtttgtccccaagaagaagtcagacatcaagtggtacggcaagtacctcaacaaccctttgggacgcaccgtgatgttaacggttcagttcactctcggctggccgttgtacttagccttcaacgtctcgggaagaccttacgacggcggcttcgcttgccatttccaccccaacgctcccatctacaacgaccgcgagcgtctccagatatacatctccgacgctggcatcctcgccgtctgctacggtctcttccgttacgccgccgcgcagggagtggcctcgatggtctgcttctacggagtcccgcttctgattgtcaatggtttcctcgtgttgatcacttacttgcagcacacgcatccttccctgcctcactacgattcgtccgagtgggattggttgaggggagctttggctaccgttgacagagactacggaatcttgaacaaggtcttccacaatattaccgacacgcacgtggcgcatcatctgttctccacgatgccgcattatcacgcgatggaagctaccaaggcgataaagccgatactgggagagtattatcagttcgatgggacgccggtggttaaggcgatgtggagggaggcgaaggagtgtatctatgtggaaccggacaggcaaggtgagaagaaaggtgtgttctggtacaacaataagttatga

SEQ ID NO: 3 - DNA, 1141 bp, Brassica napus
atgggcgcaggtggaagaatgcaagtctctcctccctccagctcccccggaaccaacaccctcaaacgcgtcccctgcgagacaccaccattcactctcggagacctcaagaaagcaatcccacctcactgcttcaaacgctccatcccacgctccttctcctcttcgacatcatcatctcctcctcggctcctccctctaccacctctccacagcctacttccctctcccttacctcgcctgacccctctactgggcctgccaaggctgcgtcctaacgggcctctgggtcatagcccacgagtgcggccaccacgccttcagcgaccaccagtggctggacgacgccgccggcctcgtcttccactccttcctcctcgtcccgtacttctcctggaagtacatccatgacgccaccattccaacaccggatccctcgatagggacgaagtgttcgtccccaagaagaaatccgacatcaagtggtacggcaagtacctcaacaacccgctaggacgcacggtgatgctaaccgtccagttcaagctcggctggccgttgtacttagccttcaacgtctcgggaagaccttacagcgacggtttcgcttgccatttccacccgaacgctcccatctacaacgaccgcgagcgtctccagatatacatctctgacgctggcgtcctctccgtatgttacggtctctaccgttacgctgcttcgcgaggagtagcctctgtggtctgtgtctacggagttccgcttctaattgtcaactgtttcctcgtcttgatcacttacttgcagcacacgcacccttcgctgcctcactatgattcttccgagtgggattggttgagaggagctttggctactgtggatagagactatggaatcttgaacaaggtgttccataacatcacggacacgcacgtggcgcatcatctgttctcgacgatgccgcattataacgcgatggaagcgaccaaggcgataaagccgatactttggagagtattaccagtttgatggaacgccggcggttaaggcgatgtggagggaggcgaaggagtgtatctatgttgaaccggataggcaaggtgagaagaaaggtgtgttctggtacaacaataagttatga

SEQ ID NO: 4 - DNA, 1155 bp, Brassica napus
atgggcgcaggtggaagaatgcaagtctctcctccctccagctcccccgaaaccaaaaccctcaaacgcgtcccctgcgagacaccacccttcactctcggagacctcaagaaagcaatcccacctcactgcttcaaacgctccatccctcgctccttctcctacctcctcttcgacatcctcgtctcctcctccctctaccacctctccacagcctacttccctctcctcccccaccctctcccttacctcgcctggcccctctactgggcctgccaaggctgcgtcctaacgggcctctgggtcatcgcccacgaatgcggccaccacgccttcagcgaccaccagtggctggacgacgccgtgggcctcgtcttccactccttcctcctcgtcccttacttctcctggaagtacagccatcgacgccaccattccaacaccggatccctcgagagggatgaagtgttcgtccccaagaagaaatccgacatcaagtggtacggaaagtacctcaacaacccgctaggacgcacggtgatgctaaccgtccagttcacgctcggctggccgttgtacttagccttcaacgtctctggaagaccttacagcgacggtttcgcttgccatttccacccgaacgctcccatctacaacgaccgcgagcgtctccagatatacatctctgacgctggcgtcctctccgtatgttacggtctctaccgctacgctggttcgcgaggagtggcctcgatggtctgtgtctacggagttccgcttatgattgtcaactgtttcctcgtcttgatcacttacttgcagcacacgcacccttcgctgcctcactatgattcttcggagtgggattggttgagaggagctttggctactgtggatagagactatggaatcttgaacaaggtgtttcataacatcacggacacgcacgtggcgcatcatctgttctcgacgatgccgcattataacgcgatggaagcgaccaaggcgataaagccgatacttggagagtattaccagtttgatggaacgccggtggttaaggcgatgtggagggaggcgaaggagtgtatctatgttgaaccggataggcaaggtgagaagaaaggtgtgttctggtacaacaataagttatga

SEQ ID NO: 5 - protein, 384 aa, Brassica napus
MGAGGRMQVSPPSKKSETDNIKRVPCETPPFTVGELKKAIPPHCFKRSIPRSFSYLIWDIIIASCFYYVATTYFPLLPHPLSYFAWPLYWACQGCVLTGVWVIAHECGHHAFSDYQWLDDTVGLIFHSFLLVPYFSWKYSHRRHHSNTGSLERDEVFVPKKKSDIKWYGKYLNNPLGRTVMLTVQFTLGWPLYLAFNVSGRPYDGGFACHFHPNAPIYNDRERLQIYISDAGILAVCYGLYRYAAVQGVASMVCFYGVPLLIVNGFLVLITYLQHTHPSLPHYDSSEWDWLRGALATVDRDYGILNKVFHNITDTHVAHHLFSTMPHYHAMEATKAIKPILGEYYQFDGTPVVKAMWREAKECIYVEPDRQGEKKGVFWYNNKL

SEQ ID NO: 6 - protein, 384 aa, Brassica napus
MGAGGRMQVSPPSKKSETDTIKRVPCETPPFTVGELKKAIPPHCFKRSIPRSFSYLIWDIIIASCFYYVATTYFPLLPHPLSYFAWPLYWACQGCVLTGVWVIAHECGHHAFSDYQWLDDTVGLIFHSFLLVPYFSWKYSHRRHHSNTGSLERDEVFVPKKKSDIKWYGKYLNNPLGRTVMLTVQFTLGWPLYLAFNVSGRPYDGGFACHFHPNAPIYNDRERLQIYISDAGILAVCYGLFRYAAAQGVASMVCFYGVPLLIVNGFLVLITYLQHTHPSLPHYDSSEWDWLRGALATVDRDYGILNKVFHNITDTHVAHHLFSTMPHYHAMEATKAIKPILGEYYQFDGTPVVKAMWREAKECIYVEPDRQGEKKGVFWYNNKL

SEQ ID NO: 7 - protein, 384 aa, Brassica napus; identical to SEQ ID NO: 5

SEQ ID NO: 8 - protein, 384 aa, Brassica napus; identical to SEQ ID NO: 5

SEQ ID NO: 9 - protein, 11 aa, Artificial Sequence
  Synthetic Construct
LDLNRPPPVEN

SEQ ID NO: 10 - protein, 8 aa, Artificial Sequence
  Synthetic Construct
LRLFGVNM

SEQ ID NO: 11 - protein, 8 aa, Artificial Sequence
  Synthetic Construct
LKLFGVWL

SEQ ID NO: 12 - protein, 10 aa, Artificial Sequence
  Synthetic Construct
LDLELRLGFA

SEQ ID NO: 13 - protein, 203 aa, Artificial Sequence
  Synthetic Construct
ERSNSIELRNSFYGRARTSPWSYGDYDNCQQDHDYLLGFSWPPRSYTCSFCKREFRSAQALGGHMNVHRRDRARLRLQQSPSSSSTPSPPYPNPNYSYSTMANSPPPHHSPLTLFPTLSPPSSPRYRAGLIRSLSPKSKHTPENACKTKKSSLLVEAGEATRFTSKDACKILRNDEIISLELEIGLINESEQDLDLELRLGFA

SEQ ID NO: 14 - DNA, 20 bp, Artificial Sequence
  Synthetic Construct
atcgagcgtttgaaacagtg

SEQ ID NO: 15 - DNA, 63 bp, Artificial Sequence
  Synthetic Construct
tgtaatacgactcactataggtcgagcgtttgaaacagtggttttagagctagaaatagcaag

SEQ ID NO: 16 - DNA, 20 bp, Artificial Sequence
  Synthetic Construct
atggagcgtttgaagcagtg

SEQ ID NO: 17 - DNA, 63 bp, Artificial Sequence
  Synthetic Construct
tgtaatacgactcactataggtggagcgtttgaagcagtggttttagagctagaaatagcaag

SEQ ID NO: 18 - DNA, 41 bp, Artificial Sequence
  Synthetic Construct
gaaagcaatcccaccgcacatgtttcaaacgctcgatccct

SEQ ID NO: 19 - DNA, 41 bp, Artificial Sequence
  Synthetic Construct
gaaagcaatcccaccgcacctgtttcaaacgctcgatccct

SEQ ID NO: 20 - DNA, 41 bp, Artificial Sequence
  Synthetic Construct
gaaagcaatcccaccgcacgtgtttcaaacgctcgatccct

SEQ ID NO: 21 - DNA, 41 bp, Artificial Sequence
  Synthetic Construct
gaaagcaatcccaccgcacttgtttcaaacgctcgatccct

SEQ ID NO: 22 - DNA, 39 bp, Artificial Sequence
  Synthetic Construct
gaaagcaatcccaccgcacgtttcaaacgctcgatccct

SEQ ID NO: 23 - DNA, 38 bp, Artificial Sequence
  Synthetic Construct
gaaagcaatcccaccgcactttcaaacgctcgatccct

SEQ ID NO: 24 - DNA, 41 bp, Artificial Sequence
  Synthetic Construct
gaaagcaatcccacctcacatgcttcaaacgctccatccca

SEQ ID NO: 25 - DNA, 41 bp, Artificial Sequence
  Synthetic Construct
gaaagcaatcccacctcacctgcttcaaacgctccatccca

SEQ ID NO: 26 - DNA, 41 bp, Artificial Sequence
  Synthetic Construct
gaaagcaatcccacctcacgtgcttcaaacgctccatccca

SEQ ID NO: 27 - DNA, 41 bp, Artificial Sequence
  Synthetic Construct
gaaagcaatcccacctcacttgcttcaaacgctccatccca

SEQ ID NO: 28 - DNA, 39 bp, Artificial Sequence
  Synthetic Construct
gaaagcaatcccacctcacgcttcaaacgctccatccca

SEQ ID NO: 29 - DNA, 38 bp, Artificial Sequence
  Synthetic Construct
gaaagcaatcccacctcaccttcaaacgctccatccca

SEQ ID NO: 30 - protein, 136 aa, Artificial Sequence
  Synthetic Construct
MGAGGRMQVSPPSSSPGTNTLKRVPCETPPFTLGDLKKAIPPHCFKRSIPRSFSSSTSSSPPRLLPLPPLHSLLPSPLPRLTPLLGLPRLRPNGPLGHSPRVRPPRLQRPPVAGRRRRPRLPLLPPRPVLLLEVHP

SEQ ID NO: 31 - protein, 384 aa, Artificial Sequence
  Synthetic Construct
MGAGGRMQVSPPSSSPETKTLKRVPCETPPFTLGDLKKAIPPHCFKRSIPRSFSYLLFDILVSSSLYHLSTAYFPLLPHPLPYLAWPLYWACQGCVLTGLWVIAHECGHHAFSDHQWLDDAVGLVFHSFLLVPYFSWKYSHRRHHSNTGSLERDEVFVPKKKSDIKWYGKYLNNPLGRTVMLTVQFTLGWPLYLAFNVSGRPYSDGFACHFHPNAPIYNDRERLQIYISDAGVLSVCYGLYRYAGSRGVASMVCVYGVPLMIVNCFLVLITYLQHTHPSLPHYDSSEWDWLRGALATVDRDYGILNKVFHNITDTHVAHHLFSTMPHYNAMEATKAIKPILGEYYQFDGTPVVKAMWREAKECIYVEPDRQGEKKGVFWYNNKL

SEQ ID NO: 32 - DNA, 388 bp, Brassica napus
gcaggtggaagaatgcaagtgtctcctccctccaaaaagtctgaaaccgacaacatcaagcgcgtaccctgcgagacaccgcccttcactgtcggagaactcaagaaagcaatcccaccgcactgtttcaaacgctcgatccctcgctctttctcctacctcatctgggacatcatcatagcctcctgcttctactacgtcgccaccacttacttccctctcctccctcaccctctctcctacttcgcctggcctctctactgggcctgccagggctgcgtcctaaccggcgtctgggtcatagcccacgagtgcggccaccacgccttcagcgactaccagtggctggacgacaccgtcggcctcatcttccactccttcctcctcg

SEQ ID NO: 33 - DNA, 389 bp, Artificial Sequence
  Synthetic Construct
gcaggtggaagaatgcaagtgtctcctccctccaaaaagtctgaaaccgacaacatcaagcgcgtaccctgcgagacaccgcccttcactgtcggagaactcaagaaagcaatcccaccgcacttgtttcaaacgctcgatccctcgctctttctcctacctcatctgggacatcatcatagcctcctgcttctactacgtcgccaccacttacttccctctcctccctcaccctctctcctacttcgcctggcctctctactgggcctgccagggctgcgtcctaaccggcgtctgggtcatagcccacgagtgcggccaccacgccttcagcgactaccagtggctggacgacaccgtcggcctcatcttccactccttcctcctcg

SEQ ID NO: 34 - DNA, 387 bp, Artificial Sequence
  Synthetic Construct
gcaggtggaagaatgcaagtgtctcctccctccaaaaagtctgaaaccgacaacatcaagcgcgtaccctgcgagacaccgcccttcactgtcggagaactcaagaaagcaatcccaccgcacttttcaaacgctcgatccctcgctctttctcctacctcatctgggacatcatcatagcctcctgcttctactacgtcgccaccacttacttccctctcctccctcaccctctctcctacttcgcctggcctctctactgggcctgccagggctgcgtcctaaccggcgtctgggtcatagcccacgagtgcggccaccacgccttcagcgactaccagtggctggacgacaccgtcggcctcatcttccactccttcctcctcg

SEQ ID NO: 35 - DNA, 387 bp, Artificial Sequence
  Synthetic Construct
gcaggtggaagaatgcaagtgtctcctccctccaaaaagtctgaaaccgacaacatcaagcgcgtaccctgcgagacaccgcccttcactgtcggagaactcaagaaagcaatcccaccgcactgttcaaacgctcgatccctcgctctttctcctacctcatctgggacatcatcatagcctcctgcttctactacgtcgccaccacttacttccctctcctccctcaccctctctcctacttcgcctggcctctctactgggcctgccagggctgcgtcctaaccggcgtctgggtcatagcccacgagtgcggccaccacgccttcagcgactaccagtggctggacgacaccgtcggcctcatcttccactccttcctcctcg

SEQ ID NO: 36 - DNA, 386 bp, Artificial Sequence
  Synthetic Construct
gcaggtggaagaatgcaagtgtctcctccctccaaaaagtctgaaaccgacaacatcaagcgcgtaccctgcgagacaccgcccttcactgtcggagaactcaagaaagcaatcccaccgcactttcaaacgctcgatccctcgctctttctcctacctcatctgggacatcatcatagcctcctgcttctactacgtcgccaccacttacttccctctcctccctcaccctctctcctacttcgcctggcctctctactgggcctgccagggctgcgtcctaaccggcgtctgggtcatagcccacgagtgcggccaccacgccttcagcgactaccagtggctggacgacaccgtcggcctcatcttccactccttcctcctcg

SEQ ID NO: 37 - DNA, 388 bp, Brassica napus
gcaggtggaagaatgcaagtgtctcctccctccaagaagtctgaaaccgacaccatcaagcgcgtaccctgcgagacaccgcccttcactgtcggagaactcaagaaagcaatcccaccgcactgtttcaaacgctcgatccctcgctctttctcctacctcatctgggacatcatcatagcctcctgcttctactacgtcgccaccacttacttccctctcctccctcaccctctctcctacttcgcctggcctctctactgggcctgccaagggtgcgtcctaaccggcgtctgggtcatagcccacgagtgcggccaccacgccttcagcgactaccagtggcttgacgacaccgtcggtctcatcttccactccttcctcctcg

SEQ ID NO: 38 - DNA, 389 bp, Artificial Sequence
  Synthetic Construct
gcaggtggaagaatgcaagtgtctcctccctccaagaagtctgaaaccgacaccatcaagcgcgtaccctgcgagacaccgcccttcactgtcggagaactcaagaaagcaatcccaccgcacttgtttcaaacgctcgatccctcgctctttctcctacctcatctgggacatcatcatagcctcctgcttctactacgtcgccaccacttacttccctctcctccctcaccctctctcctacttcgcctggcctctctactgggcctgccaagggtgcgtcctaaccggcgtctgggtcatagcccacgagtgcggccaccacgccttcagcgactaccagtggcttgacgacaccgtcggtctcatcttccactccttcctcctcg

SEQ ID NO: 39 - DNA, 387 bp, Artificial Sequence
  Synthetic Construct
gcaggtggaagaatgcaagtgtctcctccctccaagaagtctgaaaccgacaccatcaagcgcgtaccctgcgagacaccgcccttcactgtcggagaactcaagaaagcaatcccaccgcatgtttcaaacgctcgatccctcgctctttctcctacctcatctgggacatcatcatagcctcctgcttctactacgtcgccaccacttacttccctctcctccctcaccctctctcctacttcgcctggcctctctactgggcctgccaagggtgcgtcctaaccggcgtctgggtcatagcccacgagtgcggccaccacgccttcagcgactaccagtggcttgacgacaccgtcggtctcatcttccactccttcctcctcg

SEQ ID NO: 40 - DNA, 387 bp, Artificial Sequence
  Synthetic Construct
gcaggtggaagaatgcaagtgtctcctccctccaagaagtctgaaaccgacaccatcaagcgcgtaccctgcgagacaccgcccttcactgtcggagaactcaagaaagcaatcccaccgcacgtttcaaacgctcgatccctcgctctttctcctacctcatctgggacatcatcatagcctcctgcttctactacgtcgccaccacttacttccctctcctccctcaccctctctcctacttcgcctggcctctctactgggcctgccaagggtgcgtcctaaccggcgtctgggtcatagcccacgagtgcggccaccacgccttcagcgactaccagtggcttgacgacaccgtcggtctcatcttccactccttcctcctcg

SEQ ID NO: 41 - DNA, 386 bp, Artificial Sequence
  Synthetic Construct
gcaggtggaagaatgcaagtgtctcctccctccaagaagtctgaaaccgacaccatcaagcgcgtaccctgcgagacaccgcccttcactgtcggagaactcaagaaagcaatcccaccgcactttcaaacgctcgatccctcgctctttctcctacctcatctgggacatcatcatagcctcctgcttctactacgtcgccaccacttacttccctctcctccctcaccctctctcctacttcgcctggcctctctactgggcctgccaagggtgcgtcctaaccggcgtctgggtcatagcccacgagtgcggccaccacgccttcagcgactaccagtggcttgacgacaccgtcggtctcatcttccactccttcctcctcg

SEQ ID NO: 42 - DNA, 385 bp, Artificial Sequence
  Synthetic Construct
gcaggtggaagaatgcaagtgtctcctccctccaagaagtctgaaaccgacaccatcaagcgcgtaccctgcgagacaccgcccttcactgtcggagaactcaagaaagcaatcccaccgtgtttcaaacgctcgatccctcgctctttctcctacctcatctgggacatcatcatagcctcctgcttctactacgtcgccaccacttacttccctctcctccctcaccctctctcctacttcgcctggcctctctactgggcctgccaagggtgcgtcctaaccggcgtctgggtcatagcccacgagtgcggccaccacgccttcagcgactaccagtggcttgacgacaccgtcggtctcatcttccactccttcctcctcg

SEQ ID NO: 43 - DNA, 384 bp, Artificial Sequence
  Synthetic Construct
gcaggtggaagaatgcaagtgtctcctccctccaagaagtctgaaaccgacaccatcaagcgcgtaccctgcgagacaccgcccttcactgtcggagaactcaagaaagcaatcccaccgcattcaaacgctcgatccctcgctctttctcctacctcatctgggacatcatcatagcctcctgcttctactacgtcgccaccacttacttccctctcctccctcaccctctctcctacttcgcctggcctctctactgggcctgccaagggtgcgtcctaaccggcgtctgggtcatagcccacgagtgcggccaccacgccttcagcgactaccagtggcttgacgacaccgtcggtctcatcttccactccttcctcctcg

SEQ ID NO: 44 - DNA, 382 bp, Artificial Sequence
  Synthetic Construct
gcaggtggaagaatgcaagtgtctcctccctccaagaagtctgaaaccgacaccatcaagcgcgtaccctgcgagacaccgcccttcactgtcggagaactcaagaaagcaatcccaccgcactaacgctcgatccctcgctctttctcctacctcatctgggacatcatcatagcctcctgcttctactacgtcgccaccacttacttccctctcctccctcaccctctctcctacttcgcctggcctctctactgggcctgccaagggtgcgtcctaaccggcgtctgggtcatagcccacgagtgcggccaccacgccttcagcgactaccagtggcttgacgacaccgtcggtctcatcttccactccttcctcctcg

SEQ ID NO: 45 - DNA, 374 bp, Brassica napus
gcaggtggaagaatgcaagtctctcctccctccagctcccccggaaccaacaccctcaaacgcgtcccctgcgagacaccaccattcactctcggagacctcaagaaagcaatcccacctcactgcttcaaacgctccatcccacgctccttctcctcttcgacatcatcatctcctcctcggctcctccctctaccacctctccacagcctacttccctctcccttacctcgcctgacccctctactgggcctgccaaggctgcgtcctaacgggcctctgggtcatagcccacgagtgcggccaccacgccttcagcgaccaccagtggctggacgacgccgccggcctcgtcttccactccttcctcctcg

SEQ ID NO: 46 - DNA, 375 bp, Artificial Sequence
  Synthetic Construct
gcaggtggaagaatgcaagtctctcctccctccagctcccccggaaccaacaccctcaaacgcgtcccctgcgagacaccaccattcactctcggagacctcaagaaagcaatcccacctcacttgcttcaaacgctccatcccacgctccttctcctcttcgacatcatcatctcctcctcggctcctccctctaccacctctccacagcctacttccctctcccttacctcgcctgacccctctactgggcctgccaaggctgcgtcctaacgggcctctgggtcatagcccacgagtgcggccaccacgccttcagcgaccaccagtggctggacgacgccgccggcctcgtcttccactccttcctcctcg

SEQ ID NO: 47 - DNA, 388 bp, Brassica napus
gcaggtggaagaatgcaagtctctcctccctccagctcccccgaaaccaaaaccctcaaacgcgtcccctgcgagacaccacccttcactctcggagacctcaagaaagcaatcccacctcactgcttcaaacgctccatccctcgctccttctcctacctcctcttcgacatcctcgtctcctcctccctctaccacctctccacagcctacttccctctcctcccccaccctctcccttacctcgcctggcccctctactgggcctgccaaggctgcgtcctaacgggcctctgggtcatcgcccacgaatgcggccaccacgccttcagcgaccaccagtggctggacgacgccgtgggcctcgtcttccactccttcctcctcg

SEQ ID NO: 48 - DNA, 389 bp, Artificial Sequence
  Synthetic Construct
gcaggtggaagaatgcaagtctctcctccctccagctcccccgaaaccaaaaccctcaaacgcgtcccctgcgagacaccacccttcactctcggagacctcaagaaagcaatcccacctcacttgcttcaaacgctccatccctcgctccttctcctacctcctcttcgacatcctcgtctcctcctccctctaccacctctccacagcctacttccctctcctcccccaccctctcccttacctcgcctggcccctctactgggcctgccaaggctgcgtcctaacgggcctctgggtcatcgcccacgaatgcggccaccacgccttcagcgaccaccagtggctggacgacgccgtgggcctcgtcttccactccttcctcctcg

SEQ ID NO: 49 - DNA, 387 bp, Artificial Sequence
  Synthetic Construct
gcaggtggaagaatgcaagtctctcctccctccagctcccccgaaaccaaaaccctcaaacgcgtcccctgcgagacaccacccttcactctcggagacctcaagaaagcaatcccacctcacgcttcaaacgctccatccctcgctccttctcctacctcctcttcgacatcctcgtctcctcctccctctaccacctctccacagcctacttccctctcctcccccaccctctcccttacctcgcctggcccctctactgggcctgccaaggctgcgtcctaacgggcctctgggtcatcgcccacgaatgcggccaccacgccttcagcgaccaccagtggctggacgacgccgtgggcctcgtcttccactccttcctcctcg

SEQ ID NO: 50 - DNA, 385 bp, Artificial Sequence
  Synthetic Construct
gcaggtggaagaatgcaagtctctcctccctccagctcccccgaaaccaaaaccctcaaacgcgtcccctgcgagacaccacccttcactctcggagacctcaagaaagcaatcccacctcacttcaaacgctccatccctcgctccttctcctacctcctcttcgacatcctcgtctcctcctccctctaccacctctccacagcctacttccctctcctcccccaccctctcccttacctcgcctggcccctctactgggcctgccaaggctgcgtcctaacgggcctctgggtcatcgcccacgaatgcggccaccacgccttcagcgaccaccagtggctggacgacgccgtgggcctcgtcttccactccttcctcctcg

SEQ ID NO: 51 - DNA, 389 bp, Artificial Sequence; identical to SEQ ID NO: 33
  Synthetic Construct

SEQ ID NO: 52 - DNA, 389 bp, Artificial Sequence; identical to SEQ ID NO: 38
  Synthetic Construct

SEQ ID NO: 53 - DNA, 375 bp, Artificial Sequence; identical to SEQ ID NO: 46
  Synthetic Construct

SEQ ID NO: 54 - DNA, 388 bp, Artificial Sequence; identical to SEQ ID NO: 47
  Synthetic Construct